European Patent Specification EP 3 443 103 B1, published November 12, 2025. Title: Kernkodierte mnnliche Sterilitt durch Mutation in Cytochrom P450 Oxidase. Applicant: KWS SAAT SE. The sequence listing filed with the application follows.

SEQUENCE LISTING (27 sequences)

SEQ ID NO: 1 - DNA, 4328 bp, Beta vulgaris
  Promotor (1)..(1518): putativer Promotor
  Gen (1519)..(4275)
  5'UTR (1519)..(1761)
  exon (1762)..(2679): Exon 1
  Intron (2680)..(3506)
  exon (3507)..(4142): Exon 2
  3'UTR (4143)..(4275)
ttattaaacctgattggaacttattgaaccttattagacctgattggaacttattgcacctgattggaacttattggaacttattagaccttattggaacttattgcacttattagaccttattgcaacttatctgaacttatctgaacaaatctgaacttattggacctgaaacttaattttttaagttgaacagaacgcacccttagtatatcgttgccacatgtgcgttgaatttttccttttcctatcctttccactccatattctcctcaaaagtgtgtaaaaatccgacacacgagtagaatgggattgaagtgggtcaagatctgaaaccaatgggtcaatgccacaaaataaggtaaggtttctcgcagtagcaaaaaaataaagttaagttgagagaaaaattatgaatagttgtttctcgtgaagagttgtatacaaaaaaagtctaatttgatacattttcttttacatttataaaggattgaccaatcatccaaattaccaaatatttaggatataaatctttcagattacaacccatatatgatacactaaattttacatgaggcaatggaggatttgcatgaatatcgaggagagaaaaaattagttacaaaacttgcataatttatccaaaccaaatcaagtcaagaaacaacgaacaatattatcattagtactataagtatatattataggcttagagcaaagccctaactaccacactgcacacaaatgataactagtaagagaggaaaatacaaatttaagattcaacatagcaaattattcatgattcatgattcatgattcatgattcatgattcacgaacatcaagaatggtatagctgataaaggacaatttaaacataagtgtaaagctcgcacatcatcaattatattcgcatactactagaccaatctttacttagtacatgtgttagtacatgtgttacttcatatcagatgtattgattgttgccaatgacatatcatgttcacttaatcttagggccatttaattataacatggagaataatacaacttaaaattatgtggtggctatcatctcattttctagataattaaacctttattttgtatacatatatattgtctttacatagcaaaacaatattgaaggtataacaacctttcccttttcttttactacatgtttatgttagagtttttcgatttacgattgtggtaaattaattgtaattgatcggttgtcttgtagtcaagaaatgacgtatgaatcaatttagggcatgttctcttcggcataaaacagctgaactgaattgaactgaactgaaatgaatagtgatatgtgagagtaaaagtattgtcaagagctgaactgagctgaactgaacggatctgaactgaactgatctaatctgaactaatctgaactgaactgaactgaattgaactgaaaataagctagggaaaacagacccttactactattatataacctcgtttaaatattaggaaattaaaaaaataattatatttctttatactttattaacctattgaggtttttatattgactcccaaatactattttatagatcatgccatgttaatgagcaaactactttctcacatctttataggagaaaaagtagatcactcactagcatatcatgaccagcgaaaccaaccaacgctaatagttttattgcttccattagagataagagttaactaataataccatctttgtgaaattttgatggattttggaactttagcaatatatttactgtgtgcactttttgctaccaaaattttataccaatggctcaagtcctacttatacacaacatacaaactccctcccggcccaccaaggtggcccttatttggaaacctccttcaactagggccacttccccaccgcgatttcgcctcattttgtgaaaaatatgggcctttagtctacataaggcttggtaatgtggatgccataaccactaatgatccagaaatcatacgtgagatcttagttcgacaagatgatgtatttgcgtctcgtccacataccttagccgcaacccacttggcttacaatagtggtgatgtggccttggctccaatgggaccaaaatggaaaagaatgagaaggatatgcatggagcacttgctcacaactagacgacttgaactatttgtgagtcatagggctgatgaggcacgacatttggtccaagacgtattaactcgttcccacaaagataaagttgttaatttgagggaagtgttaggtgcattttctatgaataacgtgactagaatgttgctagggaagcaatactttggggccgggacggcgggcccacaagaggctctagagtttatgcatataacacatgagttgttttggttactaggcttgatttacttgggtgattatttgcctttttggaggtgggttgatccatatggatgtgaaaagaaaatgagggaagttgaaaaaagggtagatgatttccatcgcaaaattatagaggaacataggaaggagaagaaaaggaaagaagaaatgggagtgaatgagggtgaaatggattttgtagatattttgttggctttgcctggtgaaaatggaaatgagcatatggatgatgcagatattaaagctctaattcaggtaattcatgtataatttgaatgtgatcgatacaaagtttgatagaaaacatatttgcataaatatatggttgccctactagacccaataaaatacataattattgccttactagttgaaagttgaaacaacctagctaccattttgttgtgattatcattagccaaccaaaattatttcttgcatccatatattaatgttgagatcagagtcggcatatttacaattacttgtaacattttaagcaaacaaattaaaatattttttggcaagtccattttattgaataatacctatatcttaaaatgaattcttggtcatgtacacttgcctttcaaggtaccaatatttgaccatatgtaattactattaacaaatttgataaaatctaataatatgtaaatatacattcacgcacatattagaaacaaagatcacaaatgataatgcaaaataacttatttgaactaatgttgtgaagttaaatttggaacaaaaggtatatttgtattgccgaattttaatttataaattacttataacaacaactcaatatgtaaaactgttaagatggagtgtggatagaatgagatgagtatacttttactagttaccactcgaaaatgcatttcctcctttgtttatagttgttctaacttctattatcataaataattttttggacttatttcaatgtatatttacaacgctaattgtttaattttttaaaaatacataatgtaaacaaggatttcatggtcaattatacacattataaatattatcttaaaaaacttattaatgctcaattagtatccataatataggatatgatagcagcagcaacagacacatcagctgtaaccaacgaatgggccatggcagaagtaataaaacacccacgtgtcctccacaagatccaacaagagcttaacacaatagtaggacccaatcgaatggtaacagaatcagatcttccccaccttaactacctacgttgtgtcgtacgtgaaacgttccgaatgcatccagcaggaccctttttaatcccacatgaatcactacgccatacaacaatcaacggctatgatatcccatctgggacacgtgtcttcatcaacacacatgggttaggacgtaaccttaaagtgtgggacaacatagaggatttttaccctgaaagacattggccgttggatggaagtagagttgagattagccatggatctgattttaaaatattaccatttagtgctgggaagagaagatgtcctggggccccacttggggtggtgtttgtgttgatgggattggctacactttttcatgcatttgattggttaccacctgatggaatgaaggcagaagaaattgatactaaggaagtttatgggatgactatgcctaaagctcaacctttaatggctttggctaaacctaggcttgctcatttatatctttgatacatgttcatattgtggtgcacttataagcacaatagacaaatacaagtttgtatcgactctaacatgttgtttagtattagtatactgcaactctacaagtatgtaatttctataaactataaacacaagtcataacgcattttgttttgaaaaaaaagaggttacattgtcttacaccataaa

SEQ ID NO: 2 - DNA, 1930 bp, Artificial Sequence
  cDNA-CYPgst gene (Beta vulgaris)
  5'UTR (1)..(243)
  exon (244)..(1161): Exon 1
  exon (1162)..(1797): Exon 2
  3'UTR (1798)..(1930)
ttaaaaaaataattatatttctttatactttattaacctattgaggtttttatattgactcccaaatactattttatagatcatgccatgttaatgagcaaactactttctcacatctttataggagaaaaagtagatcactcactagcatatcatgaccagcgaaaccaaccaacgctaatagttttattgcttccattagagataagagttaactaataataccatctttgtgaaattttgatggattttggaactttagcaatatatttactgtgtgcactttttgctaccaaaattttataccaatggctcaagtcctacttatacacaacatacaaactccctcccggcccaccaaggtggcccttatttggaaacctccttcaactagggccacttccccaccgcgatttcgcctcattttgtgaaaaatatgggcctttagtctacataaggcttggtaatgtggatgccataaccactaatgatccagaaatcatacgtgagatcttagttcgacaagatgatgtatttgcgtctcgtccacataccttagccgcaacccacttggcttacaatagtggtgatgtggccttggctccaatgggaccaaaatggaaaagaatgagaaggatatgcatggagcacttgctcacaactagacgacttgaactatttgtgagtcatagggctgatgaggcacgacatttggtccaagacgtattaactcgttcccacaaagataaagttgttaatttgagggaagtgttaggtgcattttctatgaataacgtgactagaatgttgctagggaagcaatactttggggccgggacggcgggcccacaagaggctctagagtttatgcatataacacatgagttgttttggttactaggcttgatttacttgggtgattatttgcctttttggaggtgggttgatccatatggatgtgaaaagaaaatgagggaagttgaaaaaagggtagatgatttccatcgcaaaattatagaggaacataggaaggagaagaaaaggaaagaagaaatgggagtgaatgagggtgaaatggattttgtagatattttgttggctttgcctggtgaaaatggaaatgagcatatggatgatgcagatattaaagctctaattcaggatatgatagcagcagcaacagacacatcagctgtaaccaacgaatgggccatggcagaagtaataaaacacccacgtgtcctccacaagatccaacaagagcttaacacaatagtaggacccaatcgaatggtaacagaatcagatcttccccaccttaactacctacgttgtgtcgtacgtgaaacgttccgaatgcatccagcaggaccctttttaatcccacatgaatcactacgccatacaacaatcaacggctatgatatcccatctgggacacgtgtcttcatcaacacacatgggttaggacgtaaccttaaagtgtgggacaacatagaggatttttaccctgaaagacattggccgttggatggaagtagagttgagattagccatggatctgattttaaaatattaccatttagtgctgggaagagaagatgtcctggggccccacttggggtggtgtttgtgttgatgggattggctacactttttcatgcatttgattggttaccacctgatggaatgaaggcagaagaaattgatactaaggaagtttatgggatgactatgcctaaagctcaacctttaatggctttggctaaacctaggcttgctcatttatatctttgatacatgttcatattgtggtgcacttataagcacaatagacaaatacaagtttgtatcgactctaacatgttgtttagtattagtatactgcaactctacaagtatgtaatttctataaactataaacacaagt

SEQ ID NO: 3 - protein, 517 aa, Beta vulgaris
  PEPTIDE (1)..(517): protein CYPgst (Beta vulgaris)
MDFGTLAIYLLCALFATKILYQWLKSYLYTTYKLPPGPPRWPLFGNLLQLGPLPHRDFASFCEKYGPLVYIRLGNVDAITTNDPEIIREILVRQDDVFASRPHTLAATHLAYNSGDVALAPMGPKWKRMRRICMEHLLTTRRLELFVSHRADEARHLVQDVLTRSHKDKVVNLREVLGAFSMNNVTRMLLGKQYFGAGTAGPQEALEFMHITHELFWLLGLIYLGDYLPFWRWVDPYGCEKKMREVEKRVDDFHRKIIEEHRKEKKRKEEMGVNEGEMDFVDILLALPGENGNEHMDDADIKALIQDMIAAATDTSAVTNEWAMAEVIKHPRVLHKIQQELNTIVGPNRMVTESDLPHLNYLRCVVRETFRMHPAGPFLIPHESLRHTTINGYDIPSGTRVFINTHGLGRNLKVWDNIEDFYPERHWPLDGSRVEISHGSDFKILPFSAGKRRCPGAPLGVVFVLMGLATLFHAFDWLPPDGMKAEEIDTKEVYGMTMPKAQPLMALAKPRLAHLYL

SEQ ID NO: 4 - DNA, 27 bp, Artificial Sequence
  s1e5983d14 Forward (Fw) Primer (5' -3')
accaaaattttataccaatggctcaag

SEQ ID NO: 5 - DNA, 23 bp, Artificial Sequence
  s1e5983d14 Reverse (Rv) Primer (5' -3')
ggccgggagggagtttgtatgtt

SEQ ID NO: 6 - DNA, 27 bp, Artificial Sequence
  s1e5983d17 Forward (Fw) Primer (5' -3')
agaaatcatacgtgagatcttagttcg

SEQ ID NO: 7 - DNA, 26 bp, Artificial Sequence
  s1e5983d17 Reverse (Rv) Primer (5' -3')
ggtatgtggacgagacgcaaatacat

SEQ ID NO: 8 - DNA, 4220 bp, Beta vulgaris
  Promotor (1)..(1353): putativer Promotor
  Gen (1354)..(3542)
  exon (1354)..(1938): verkrztes Exon 1
  Intron (1939)..(2755)
  exon (2756)..(3394): Exon 2
  3'UTR (3395)..(3542)
gtatatcgttgccacatgtgcgttgaatttttccttttcctatcctttccactccatattctcctcaaaagtgtgtaaaaatccgacacacgagtagaatgggattgaagtgggtcaagatctgaaaccaatgggtcaatgccacaaaataaggtaaggtttctcgcagtagcaaaaaaataaagttaagttgagagaaaaattatgaatagttgtttctcgtgaagagttgtatacaaaaaaagtctaatttgatacattttcttttacatttataaaggattgaccaatcatccaaattaccaaatatttaggatataaatctttcagattacaacccatatatgatacactaaattttacatgaggcaatggaggatttgcatgaatatcgaggagagaaaaaattagttacaaaacttgcataatttatccaaaccaaatcaagtcaagaaacaacgaacaatattatcattagtactataagtatatattataggcttagagcaaagccctaactaccacactgcacacaaatgataactagtaagagaggaaaatacaaatttaagattcaacatagcaaattattcatgattcatgattcatgattcatgattcatgattcacgaacatcaagaatggtatagctgataaaggacaatttaaacataagtgtaaagctcgcacatcatcaattatattcgcatactactagaccaatctttacttagtacatgtgttagtacatgtgttacttcatatcagatgtattgattgttgccaatgacatatcatgttcacttaatcttagggccatttaattataacatggagaataatacaacttaaaattatgtggtggctatcatctcattttctagataattaaacctttattttgtatacatatatattgtctttacatagcaaaacaatattgaaggtataacaacctttcccttttcttttactacatgtttatgttagagtttttcgatttacgattgtggtaaattaattgtaattgatcggttgtcttgtagtcaagaaatgacgtatgaatcaatttagggcatgttctcttcggcataaaacagctgaactgaattgaactgaactgaaatgaatagtgatatgtgagagtaaaagtattgtcaagagctgaactgagctgaactgaacggatctgaactgaactgatctaatctgaactaatctgaactgaactgaactgaattgaactgaaaataagctagggaaaacagacccttactactattatataacctcgtttaaatattaggaaattaaaaaaataattatatttctttatactttattaacctattatacaatagtggtgatgtggccttggctccaatgggaccaaaatggaaaagaatgagaaggatatgcatggagcacttgctcacaactagacgacttgaactatttgtgagtcatagggctgatgaggcacgacatttggtccaagacgtattaactcgttcccacaaagataaagttgttaatttgagggaagtgttaggtgcattttctatgaataacgtgactagaatgttgctagggaagcaatactttggggccgggacggcgggcccacaagaggctctagagtttatgcatataacacatgagttgttttggttactaggcttgatttacttgggtgattatttgcctttttggaggtgggttgatccatatggatgtgaaaagaaaatgagggaagttgaaaaaagggtagatgatttccatcgcaaaattatagaggaacataggaaggagaagaaaaggaaagaagaaatgggagtgaatgagggtgaaatggattttgtagatattttgttggctttgcctggtgaaaatggaaatgagcatatggatgatgcagatattaaagctctaattcaggtaattcatgtataatttgaatgtgatacaaagtttgatagaaaacatatttgcataaatacatggttaccctactagacccaataaaatacataattattgccttgctagttgaaagttgaaacaacctagctaccattttgttgtgattatcattagccaaccaaaactatttcttgcatccatatattaatgttgagagtcgccatatttacaattacttgtaacattttgagcaaacaaattaaaatattttttggcaagtccattttattgaatgatacctatatcttaaaatgaatccttggttatgtacacttgcctttcaaggtaccaatatttgaccatatgtaattactattaacaaatttgataaaatctaataatatgtaaatatacgttcacgcacatattagaaacaaagatcacaaatgataatgcaaaataacttatttgaactaatgttgtgaagttaaatttggaacaaaaggtatatttgtattgccgaattttaatttataaattacttataacaacaactcaatatgtaaaactgttaagatggagtgtggatagaatgagatgagtatacttttactagttaccactcgaaattgcatttcctcctttgtttatagttgttctaacttctattatcataaataatttttggacttatttcaatgtatatttacaacgttaattgtttaattttttaaaaatacataatgtaaacaaggatttcatggtcaattatacacattatagatattatcttaaaaaacttactaatgctcaattagtgtccataatataggatatgatagcagcagcaacagacacatcagctgtaaccaacgaatgggccatggcagaagtaataaaacacccacgtgtcctccacaagatccaacaagagcttaacacaatagtaggacccaatcgaatggtaacagaatcagatcttccccaccttaactacctacgttgtgtcgtacgcgaaacgtttcggatgcatccagcaggaccctttttaatcccacatgaatcactacgccatacaacaatcaacggctatgatatcccatctgggacacgtgtcttcatcaacacacatgggttaggacgtaaccttaaagtgtgggacaacatagaggatttttaccctgaaagacattggccgttggatggaagtagagttgagattagccatggatctgattttaaaatattaccatttagtgctgggaagagaagatgtcctggggccccacttggggtggtgtttgtgttgatgggattggctacactttttcatgcatttgattggttaccacctgatggaatgaaggcagaagaaattgatactaaggaagtttatgggatgactatgcctaaagctcaacctttaatggctttggctaaacctaggcttgctcctcatttatatctttgatacatgttcatattgtggtgcacttataagcacactagctcaaatagacaaatacaagcttgtattgactctaacatgttatttaatattagcatactgcaactctacaactacaagtatgtaatctctataaattataaacataagtcataacgcatcttgttttgaaaaaaaaagctacactttcttacaccataaactgttccgttactaaattcttcttggcttattttagaattaatttttcaattttcctatttacttataacacaagataagaaaatcgactaacaatatttcacaacattatatcttgatagttcgttgaaattaataattttcaataatttcaaaacgcaaaaagcttctttgttcggataaattcacgtcattttcaataaaatcgcaaaatcttcccttgccatcaaggaacaaatttttcacatcaaaactcttcttccaaaaagtatacttctccattgattatgtaaaagagtttgcatgttctaatccattagtatgtatttttcggataagaagttgtattacaagcttaaataaagatataaacttagttaaatatcgaccaatccacaatatgtatcttcatatgtgtccatcagcgcctaaccttgagatgtagatcatctaaagcacattaacatggcgtactcctcctgttcaaatcagggttgtttgaaaccaaacttctccaaaatacttcctcagtaatgaagagaaaaactcacattctgaaaaacatcaacatcatggttctatggtctagtggttatgacactggactctgaatccagtaacccgagtt

SEQ ID NO: 9 - DNA, 4068 bp, Zea mays
  exon (2001)..(2927): Exon 1
  Intron (2928)..(3017): Intron
  exon (3018)..(3683): Exon 2
gagtgtggtgcgttggttttgtcagatgtcacaggaaggatgcagacctaataccgctgcttttagttgtttgctgagtgctttggctagcctggctatgctgaatcagggattgcaagctcatgcttatgcagtcaacatgggatggatatttgactcagctgtccatgcttctttggtgacaatgtatgcaaaatgtggtaggttggctgaggctcatcgtgttttctcatgcattagaaatccaagccttgttgccattaattctatgatttcagcatttgcacaacatggcttggctgaagatgcactcaaactttttaacagaatgcaatatgatggccaaaggcctaatcatgtgacattcttgggaatactgactgcatgtgctcgagctggtttggttcaacaaggctataactactttgaatctatgagatcagtctatggcattcaaccaaaccctgaccactacacatgtatggttaatcttttaggccatgcaggcttccttgatgaagcattggaaatgattaattcgatgccccagaaagattatcctgatgcatgggcagctttgcttagctctagtagcctccattctaatcttgatttagcaaaactagcagcacagaggcttcttgagatagatccttatgacacaacagcttacagggtcctgacaaacatgttctcctcagcagggttgaagggagatgaagagatggtaaaagttgcacaattgtccaacatggctagtaagaggcctgggtatagcctcatcatacaggataagactacagaaaataactagcccaaaatgagcacttccatttacagataactggcatgtcataactcataagacagggatattgggttcacagaaaacaattctagcgccaagatgagatatcaatttgttgatgtatgctagtgcagagtcagttttagtacttaagaactgagaatgaggaatatctgataaggtgactagtgatttgaagaataaagagccaggtggtctggatcaaattttggttagtcttgcctcttatatcactgtttccaggatagaattttcagtactgcaactgatgttgtatttgaataatggaaaatattttttctccctgtaaacaatagttttgtcagatgtaaatcttatccacagtagaatatgatgccatataatgctgttcagattcattacaatcgtgaagtttattgcgcctttttcagagactggagagttgatgacacttctgcaaataattcatctgctactgttgttgaacaacaagaaaatcattggttgctgcatgctttcaagaatattttgctgcgtgatctatctattctcctcatcaattgatagagaagagtcgctgagagaggtaatctttatgcttattcattcatttcgatgagacaaccataccaaggtgaattgggtgatccctaggtctaggcttttcttttagcaatagaagcttccaagtaattcatggaggtctaaggatgttctcctcaagaaaaatagggattgtctgtgtctttgttatagatgtggcaggtggagtaggactatggtaaacaagggttttctcttatttttggctgagaaattgtagattagtggggaaactatcctaattatggcaacataatgtcagcttgctttttgattaatagtcatgtttcatgacctttttttgttctagtcctcttctttttttttccttggcattttcccagtgatctacagtttacattgcgcaagtcatgtcaagatcatgacagtttttatatacatggtggtagttgagatgcttaaccatacacatcaacacaaaaaccatgaccaatctaatactgtaaccaatttgcttcaacctcagtggctcaatttacttagtacttaagcgaagaagcttgagacgtcccataaataggccagcatttgcaatccaactttagctgccatctgtttctgaaccatggatccatttgttctctccatcctcttatgctcatcgatctttgttgtagtgtactggagaaggctgaacagcatgaggctaagacttccaccgggacctccaacatggccaattttcggcaatcttctccagttgagccctcttccccacaaagactttgcccaattttgcaccaaatatggccctctcgtctatcttcgcctgggaaccatcgatgccatcaccactgatgaccccgaagtgatccgtgaaatactcatccggcaagatgaggtctttgcttcgcggcctcggacactggctgccgtccatctcgcctatgggtgtggtgatgtggctctagctccactgggacccaactggaaaaggatgaggagagtttgcatggagcacttgctgacgaccaggcggctcgagtctttcgctgctcaccgagctcaggaggccgagcacctctgccagtttgtgtgggctaaatctcagtccgggaagcccgtgaacctcagagaggttctcggtgccttctcgatgaacaacgtcacgcggatgctgctggggaagcagtactttgggatccagtcggcaggccccggcgaggcaatggagttcatgcacatcacccacgagctgttcttcctgctgggcctgatctatctcggggactacttgccggcttggaggtgggtcgacccgtacgggtgtgagaagaggatgagggaggtggagaagaaggtggacgacttccaccagaagatcattgatgagcacaggagagctagggaggccaggaagagtcgttcctccgttgaggaagatggcggcaacggcaaagatgagatggacttcgtcgatgtgctgttatctttgcctggtgagaacgggaaggagcacatggacgacatggagatcaaagcgttgatgcaggtgtgtgtatgtgtatgctttgctattgcataccctggaattcaattcattttgttgaagctagttattatgagtaatacttcttggcaggacatgatcgctgctgctactgatacttcatcggtgacgaacgagtgggtgatggcggaggtaatcaagaacccgcgcgtgctccggcgcgtccaggaggagctggacgcggtggtggggcgcgaccggatggtggcggagtcggacctggcccacctcccctacctccggtgcgtggtgcgcgagtcattccggatgcacccggcggggccgttccttatcccgcacgagtcgctgaaggcgacgaccatcatggggtaccacgtgccggcgcgcacgcgcgtgttcatcaacacgcacgcgctggggcggaacccgcgcgtgtgggactccgtgggcgagttccggccggagcggcacctgccggcggaggagggggcgcgggtggagatcagccacctgccggacttcaagatcctgccgttcagcgccgggaagcgcaagtgccccggcgcgccgctgggcgtggcgctggtgctcatggcgctcgccaggctcttccactgcttcgactggtccccgcccgacggcctccgccccgaggacgtggacacccgggaggtgtacggcatgaccatgcccaaggccacgcccctcgtcgccgtcgccactccgcgcctgccgccgcacttgtacggcggcggcggcggcagctcggctccttagttcgatgacactttgacgcacgtgcgctgcactgccagtctcattagtcattatacgcatgatgtacttccctccatatacaatacaccgcataaaccaaacgatgaatgaaatgtagtcgttctatggtttcaatatgagaagatataattgatggttaacatcatttccctccgtttagtgataagccatatactctaggtatgtagtagtgtaacaatgcgatcccagcccaggtaacgaggtagcagagaggtgagctagctgtagctggcgacgaagcgaagcattaaacggttgcaacggcagctagccgtggcgttcatgcacggtatggccaaaaaaaagggaccctatccatctgccagttttggcgtaccaatgc

SEQ ID NO: 10 - DNA, 1593 bp, Artificial Sequence
  c-DNA CYPgst gene (Zea mays)
atggatccatttgttctctccatcctcttatgctcatcgatctttgttgtagtgtactggagaaggctgaacagcatgaggctaagacttccaccgggacctccaacatggccaattttcggcaatcttctccagttgagccctcttccccacaaagactttgcccaattttgcaccaaatatggccctctcgtctatcttcgcctgggaaccatcgatgccatcaccactgatgaccccgaagtgatccgtgaaatactcatccggcaagatgaggtctttgcttcgcggcctcggacactggctgccgtccatctcgcctatgggtgtggtgatgtggctctagctccactgggacccaactggaaaaggatgaggagagtttgcatggagcacttgctgacgaccaggcggctcgagtctttcgctgctcaccgagctcaggaggccgagcacctctgccagtttgtgtgggctaaatctcagtccgggaagcccgtgaacctcagagaggttctcggtgccttctcgatgaacaacgtcacgcggatgctgctggggaagcagtactttgggatccagtcggcaggccccggcgaggcaatggagttcatgcacatcacccacgagctgttcttcctgctgggcctgatctatctcggggactacttgccggcttggaggtgggtcgacccgtacgggtgtgagaagaggatgagggaggtggagaagaaggtggacgacttccaccagaagatcattgatgagcacaggagagctagggaggccaggaagagtcgttcctccgttgaggaagatggcggcaacggcaaagatgagatggacttcgtcgatgtgctgttatctttgcctggtgagaacgggaaggagcacatggacgacatggagatcaaagcgttgatgcaggacatgatcgctgctgctactgatacttcatcggtgacgaacgagtgggtgatggcggaggtaatcaagaacccgcgcgtgctccggcgcgtccaggaggagctggacgcggtggtggggcgcgaccggatggtggcggagtcggacctggcccacctcccctacctccggtgcgtggtgcgcgagtcattccggatgcacccggcggggccgttccttatcccgcacgagtcgctgaaggcgacgaccatcatggggtaccacgtgccggcgcgcacgcgcgtgttcatcaacacgcacgcgctggggcggaacccgcgcgtgtgggactccgtgggcgagttccggccggagcggcacctgccggcggaggagggggcgcgggtggagatcagccacctgccggacttcaagatcctgccgttcagcgccgggaagcgcaagtgccccggcgcgccgctgggcgtggcgctggtgctcatggcgctcgccaggctcttccactgcttcgactggtccccgcccgacggcctccgccccgaggacgtggacacccgggaggtgtacggcatgaccatgcccaaggccacgcccctcgtcgccgtcgccactccgcgcctgccgccgcacttgtacggcggcggcggcggcagctcggctccttag

SEQ ID NO: 11 - protein, 530 aa, Zea mays
  PEPTIDE (1)..(530): protein CYPgst (Zea mays)
MDPFVLSILLCSSIFVVVYWRRLNSMRLRLPPGPPTWPIFGNLLQLSPLPHKDFAQFCTKYGPLVYLRLGTIDAITTDDPEVIREILIRQDEVFASRPRTLAAVHLAYGCGDVALAPLGPNWKRMRRVCMEHLLTTRRLESFAAHRAQEAEHLCQFVWAKSQSGKPVNLREVLGAFSMNNVTRMLLGKQYFGIQSAGPGEAMEFMHITHELFFLLGLIYLGDYLPAWRWVDPYGCEKRMREVEKKVDDFHQKIIDEHRRAREARKSRSSVEEDGGNGKDEMDFVDVLLSLPGENGKEHMDDMEIKALMQDMIAAATDTSSVTNEWVMAEVIKNPRVLRRVQEELDAVVGRDRMVAESDLAHLPYLRCVVRESFRMHPAGPFLIPHESLKATTIMGYHVPARTRVFINTHALGRNPRVWDSVGEFRPERHLPAEEGARVEISHLPDFKILPFSAGKRKCPGAPLGVALVLMALARLFHCFDWSPPDGLRPEDVDTREVYGMTMPKATPLVAVATPRLPPHLYGGGGGSSAP

SEQ ID NO: 12 - DNA, 4880 bp, Solanum tuberosum
  exon (1762)..(2032): Exon 1
  Intron (2033)..(2448): Intron 1
  exon (2449)..(3161): Exon 2
  Intron (3162)..(4031): Intron 2
  exon (4032)..(4694): Exon 3
ataataaatattttttttaaaaaaagagagggttgttagttgcaagggtataagtgagcaaaaaggtggatggaaggataattttagaccaaaaagatgagtagaagggtatttttagaccaaaagatggatgaaggatatttttagaccatttcctgtatttcagaggtatttttggcccttttccgtatgaaaatttgaggttgtatttaagttcaattggtcaaattaataagtatttttaagactgtcaaaaatttagaaataaaactaataattcacatcaattctacaaatatttctttttaatatatagacattcggttcaagtaaaatattttaagtttttatttaatttcttgtttgtttgattatggattgccttggattctatttgcgtaatggaaatggcagctcttttcagtgtaggattggacaagttagcttggattttttttcacctactctacaaaaagtgatggggcgtccaccaaccatacgtcaacaactttgtccattctttgtacacactaccatcacaatctatcaaaagatttgttctttagtctcgtttaacatattctttcgttttcattttaatttatttgtcttatttttttttataaaataaaataaatattttttgatataatacataaatatattctttaatttcatttcatttaacatctctatactttaacttgggagtcgagtgattgggttggaagtcaggtcgtgattagaggttaggagttaggtcccaactcggaattgagattagaggtccagattagatctcaggttagagtcgggagttgggtcttaagttgtggtcaggatttgggtcctagttgaggtcacaagtcaggtccccgctcgagatcgaaaattaggtcccgagttgagatagaaagttttttgatcaagattgaggtcgtagtcaagagtcgagttctgagtcgggattgtaatcgggagtgggtccttacaggttagggcgggggtcgaaagtcgggtctcaagttaggactcgtttgagggtggtgaggtttaagtaggggtgtgcatcgatcggttcggtttatcgattttcagtttttaaatatgctaaattaataaccaaatcaaaaggttttttttatcgattttggtcattaatgactcgattttctatttaaccaattagaaaatgctcataaaacaaatagatgacttctctaacaaaatttgaccgacaagacaagacaataatgtgattattattttaggttttgacgttttgtataatgtgaagtgtgaattgaaggtttaagggcaaagacagtaactagtaatatattgagattaatatttatgtaataagtaaaagaagtaaattactggagtataatcttattgagttattgttttacccaataacacaatattaaaaatcaatatcgaatcgataacccgatattttttttaaaaaaaaattgttaacccaattgatgcatttttttatatattcgtaaaatgcgtaaattgcattaaattattcccataaataaaaaagaaacttgttcataaattcaaacttattgtgcaaattgaggaagcaaaaaagtgtgatttcaagattaatacttatagttgaaacatgtcaagatgatgggcttcctaatcgctccaaaaaaagattataaattagaattaaacatatttccttattaagcctttgtaaactacttctttcttttttttgacaaataattaaagatgattgacttgactagttttgttattgtccttctttgcacgtatcttcttaatttgatcaattatagtatagtcctttttggcgcatatcttatttccaagctacttcatttttcattcgtcgataagtcgaatcgagaaatcaatcaactccctcctggtccaaaacaatggcctattgtaggcaacctttttcagttagggcaattacctcatcgagacatggcgtctttctgcgaaaaatatggcccattggtctatctccgactaggtaatgttgatacaataaattcacaaatgaccacaatttagtccttgtaattaataaatagtcattgttttcgagtttcaaatttataagggaaacttcaagtacacttgacttggagattcacttatggatgttgcaactcgatgaacaattactattttacaaaaaaatgatcgaaaagtgataagtgataagtgataagtgaacgttatttctcatataaagttcaatgctatacagattcggtcaaactcagtaaattttacctaagtactttatccatgttaagaaaaaatcattatatatgtacacacattaaattttaaaccgagttattagcactagaatttatcgttctaacattttgaacccataaagttgatatcgtgactccaccttttgttttctcttaaaaggtaatgttgatgctatcaccaccaatgatccagaaatcataagagaaatacttgtacaacaagatgatgtttttgcatctaggccaagaactcttgctgccattcatctagcttatggttgtggggatgtggcattggctcctttaggtccaaaatggaaaagaatgagaagaatatgtatggaacatttattgacaactaaaagacttgaatcatttgcaaaacatagggcagatgaagcccaaagtctagttaaagatatttggaccaaagcccaaaaaggacaaatagtgaatttgagggaagttttgggtggattttcaatgaataatgtgactagaatgttgttaggtaaacaatattttggggcagaatcagcaggtccacaagaagcaatggaatttatgcatgtaacacatgagttattttggttacttggagtgatatatttaggtgattatttacctttttggaggtggattgatccttatggttgtgagaaaaaaatgagggatgttgaaaaaaggattgatgattttcatatgagaataattgaagaacatagaaagaagaaaggtaataaaaataataataatattgatgatgatgaaatggactttgtggatgttttattgtctctaccaggagaagatgaaggagatggtaatggaaaacaaaatatggatgatgtagagattaaagctctaattcaggtctaattttttttatatataccaactttctacctatttaatatgtcaatgcatttatctcaaactacttatatatatatccaatatatatgcatttggtgagcaacaactaccacccatgggatttctaagcttgattaacagaggttgtggtgaagtgataagtacttcttcatccctaactagaggtcttgggttcgagtcttgctggatacaaagtcgtctttgttaaagagtgttaccccataatgtgagactttccggcacgaatcaaaattttgttggaatctaatggggtatcgaacaccagttgagaaaagaaagagaagaagaaattcctacaatgtgggactttcgggagcgaacccaaattttgttggactctaatgagggtatgggacacccgtagaaaaaaaaagaaataaattcacaagtttgattgatacttaaaacataaaatttaagttatatatactgatagagtaaaacaaattacattattagtccaatttaatcggtactaccatgttattactctattaaattattatatgagacttaatatagagagttacatgtcaacttgatagtgtagacatttttagactattcatgcacaaaaacttaactctaatacaatcaatttccttgcaacttttatattagagaatatatatatatatatatatatatatatatatatagtacagtatattttaacatgtataaacaagatgcctattttattttcagcttattactaatcacaatatatatttgctacatcaatagtataaaaaaaagctaaatatggttcttttttctgctgtgacttatttcttttctttaattaaattataggatatgatagctgcagccacagacacttctgctgtgaccaacgaatgggcaatggctgaggtaatcagacatccacatgtcctcaaaaagatccaagaagaactcgatatagttgtcgggtcgggtcggatggtaaccgaatccgacttgatccatctcaagtacctccgttgtgtagtacgtgaaacattccgaatgcaccctgcgggtccattcctaatcccacatgaatcaattcgcgatactatgatcaacggctattacatcccggccaagacacgcgtgttcatcaacacacatggtcttggccggaacacaaagatttgggacaacatagatgagtttaggccagagagacatttaccaccaaatgatgatgaaaaaaacatgatcatgactactagtagtagtagagttgagattagtcatggtccagatttcaagattttgccatttagtgctggaaaaaggaagtgtcctggtgcaccattgggtgtgaaattggtgcttatggcattggctaggttgtttcattgctatgattggagtccaccaaatggagtaaagcatcaagatattgacacaaatgaagtttatggaatgactatgcctaaagctaagccattgatggctattgctaaacctagactgcctgctcacttgtaccaataattagttactagtactcaaatcaaagggaattggtctttaatggctttcgtaacgaatcaaataaagagaaatttctatttgtacctcgtaaaaaaaagctctcgcctcctgtaatagtatacttcaacatttttctcacctgtggcaatccacacagcagacttaagtctgtctgattacatagta

SEQ ID NO: 13 - DNA, 1656 bp, Artificial Sequence
  cDNA CYPgst gene (Solanum tuberosum)
atgattgacttgactagttttgttattgtccttctttgcacgtatcttcttaatttgatcaattatagtatagtcctttttggcgcatatcttatttccaagctacttcatttttcattcgtcgataagtcgaatcgagaaatcaatcaactccctcctggtccaaaacaatggcctattgtaggcaacctttttcagttagggcaattacctcatcgagacatggcgtctttctgcgaaaaatatggcccattggtctatctccgactaggtaatgttgatgctatcaccaccaatgatccagaaatcataagagaaatacttgtacaacaagatgatgtttttgcatctaggccaagaactcttgctgccattcatctagcttatggttgtggggatgtggcattggctcctttaggtccaaaatggaaaagaatgagaagaatatgtatggaacatttattgacaactaaaagacttgaatcatttgcaaaacatagggcagatgaagcccaaagtctagttaaagatatttggaccaaagcccaaaaaggacaaatagtgaatttgagggaagttttgggtggattttcaatgaataatgtgactagaatgttgttaggtaaacaatattttggggcagaatcagcaggtccacaagaagcaatggaatttatgcatgtaacacatgagttattttggttacttggagtgatatatttaggtgattatttacctttttggaggtggattgatccttatggttgtgagaaaaaaatgagggatgttgaaaaaaggattgatgattttcatatgagaataattgaagaacatagaaagaagaaaggtaataaaaataataataatattgatgatgatgaaatggactttgtggatgttttattgtctctaccaggagaagatgaaggagatggtaatggaaaacaaaatatggatgatgtagagattaaagctctaattcaggatatgatagctgcagccacagacacttctgctgtgaccaacgaatgggcaatggctgaggtaatcagacatccacatgtcctcaaaaagatccaagaagaactcgatatagttgtcgggtcgggtcggatggtaaccgaatccgacttgatccatctcaagtacctccgttgtgtagtacgtgaaacattccgaatgcaccctgcgggtccattcctaatcccacatgaatcaattcgcgatactatgatcaacggctattacatcccggccaagacacgcgtgttcatcaacacacatggtcttggccggaacacaaagatttgggacaacatagatgagtttaggccagagagacatttaccaccaaatgatgatgaaaaaaacatgatcatgactactagtagtagtagagttgagattagtcatggtccagatttcaagattttgccatttagtgctggaaaaaggaagtgtcctggtgcaccattgggtgtgaaattggtgcttatggcattggctaggttgtttcattgctatgattggagtccaccaaatggagtaaagcatcaagatattgacacaaatgaagtttatggaatgactatgcctaaagctaagccattgatggctattgctaaacctagactgcctgctcacttgtaccaataa

SEQ ID NO: 14 - protein, 551 aa, Solanum tuberosum
  PEPTID (1)..(551): protein CYPgst (Solanum tuberosum)
MIDLTSFVIVLLCTYLLNLINYSIVLFGAYLISKLLHFSFVDKSNREINQLPPGPKQWPIVGNLFQLGQLPHRDMASFCEKYGPLVYLRLGNVDAITTNDPEIIREILVQQDDVFASRPRTLAAIHLAYGCGDVALAPLGPKWKRMRRICMEHLLTTKRLESFAKHRADEAQSLVKDIWTKAQKGQIVNLREVLGGFSMNNVTRMLLGKQYFGAESAGPQEAMEFMHVTHELFWLLGVIYLGDYLPFWRWIDPYGCEKKMRDVEKRIDDFHMRIIEEHRKKKGNKNNNNIDDDEMDFVDVLLSLPGEDEGDGNGKQNMDDVEIKALIQDMIAAATDTSAVTNEWAMAEVIRHPHVLKKIQEELDIVVGSGRMVTESDLIHLKYLRCVVRETFRMHPAGPFLIPHESIRDTMINGYYIPAKTRVFINTHGLGRNTKIWDNIDEFRPERHLPPNDDEKNMIMTTSSSRVEISHGPDFKILPFSAGKRKCPGAPLGVKLVLMALARLFHCYDWSPPNGVKHQDIDTNEVYGMTMPKAKPLMAIAKPRLPAHLYQ

SEQ ID NO: 15 - protein, 525 aa, Triticum aestivum
  PEPTID (1)..(525): protein CYPgst (Trticum aestivum)
MDPFLLSIILCSCIFAAVSWKKLNGMRLRLPPGPPRWPIFGNLLQLSPLPHKDFARFCTKYGPLVYLRLGTIDAITTDDPEVIREILIRQDEVFASRPRTLAAVHLAYGCGDVALAPLGPNWKRMRRVCMEHLLTTRRLESFAAHRAEEAEHLCEFVWAKSQSGKPVNLREVLGAFSMNNVTRMLLGKQYFGLQSAGPGEAMEFMHITHELFFLLGLIYLGDYLPAWRWLDPYGCEKKMREVEKKVDDFHQKIIDEHRKARDVRKSGASLDDDGDDSKEGMDFVDVLLSLPGENGNEHMDDVEIKALMQDMIAAATDTSSVTNEWVMAEVIKNPRVLRKIQEELDAVVGTSRPHGGGGGPPPPDVPPLRRPGVLPDAPGGAIPDPARVTQGDDHHGLRHPGADEDLHQHPRAGPEPAHLGRRRRVPPREAPPGGRRARGDQPPAGLQDPALQRRQAQVPRGAAGRDPGAHGARQALPLLRLVPARRPPPRGHRHRRGLRDDHAQGQAAHRRRSTAPAAADVRLLS

SEQ ID NO: 16 - protein, 518 aa, Helianthus annuus
  PEPTID (1)..(518): protein CYPgst (Helianthus annuus)
MDLQSFISVLAFIVASRIILLWYVKQRVTQNTTHRLPPGPPRWPIVGNLLQLGPLPHRDLASFCERYGPLVYLRLGKVDAITTNDPNIIREILVKQDDVFASRPQTLAAVHLAYNCGDVALAPFGPRWKWMRRICMEQLLTTKRLESFAKQRASEAQHLVQDVWALSQANGPINLREVLGGFSMNNVTRMLLGKQYFGSGSAGPKEATEFMHITHELFWLLGLIYLGDYLPFWRWIDPYGCEKKMREVEKRVDDFHMKIIEEHRQRRKNGEQKDEGIMDFVDVLLSLPGEDGKDHMDDRQIKALVQDMIAAATDTSAVTNEWAMAEVIKHPHVLRKIQEELDNVVGPDRMVSESDLSNLNYLRCVVRETFRMHPAGPFLIPHESLRATEINGYYIPAKTRVFINTHGLGRNTVLWDDINVFRPERHLTSDGSRVEISHGDDFKILPFSAGKRKCPGAPLGVTLVLMALARLFHCFDWSPPDGLKCEDIDTQEIYGMTMPKAKPLMAVAKPRLASYMYQ

SEQ ID NO: 17 - protein, 530 aa, Hordeum vulgare
  PEPTID (1)..(530): protein CYPgst (Hordeum vulgare)
MDLFLFSIILCSCIFAAVSWRKLSRLRLRLPPGPPRWPIFGNLLQLSPLPHKDFARFCTKYGPLVYLRLGTIDAITTDDPEVIREILVRQDEVFASRPRTLAAVHLAYGCGDVALAPLGPNWKRMRRVCMEHLLTTKRLESFAAHRAQEAEHLCEFVWAKSQSGKPVNLREVLGAFSMNNVTRMLLGKQYFGLQSAGPGEAMEFMHITHELFFLLGLIYLGDYLPAWRWVDPYGCEKKMREVEKKVDDFHQKIIDEHRKARDARKSAASLDDGDDSKEDMDFVDVLLSLPGENGNEHMDDVEIKALMQDMIAAATDTSSVTNEWVMAEVIKNPCVLRKIQEELDAVVGRSRMVVESDLPHLTYLRCVVRESFRMHPAGPFLIPHESLKATTIMGYDIPAQTRIFINTHALGRNPRIWDDVGEFHPERHLPADGGRVEISHLPDFKILPFSAGKRKCPGAPLGVILVLMALARLFHCFDWSPPDGLRPEDIDTDEVYGMTMPKAKPLIAAVQPRLPPQMYGSCPSHGMQMQ

SEQ ID NO: 18 - protein, 466 aa, Brassica napus
  PEPTID (1)..(466): protein CYPgst (Brassica napus)
MAALCSKYGPLVYLRLGNIDAITTNDPETIREILFRQDDVFASRPKTLAAVHLAYGCGDVALAPMGPHWKRMRRICMEHLLTTKRLESFTSQRAEEAQYLIQDVCKRAECGKPINLREVLGAFSMNNVTRMLLGKQFFGPGSVVGAKEAQEFMHITHKLFRLLGVIYLGDYLPFWRWVDPYGCEKEMRDVEKRVDKFHTKIIEEHRRAKREKEDKNIEGDMDFVDVLLSLPGENGKEHMDDVEIKALIQDMIAAATDTSAVTNEWAMAEVIKQPRVMRKIQEELDNVVGSNRMVNETDLVHLNYLRCVVRETFRMHPAGPFLIPHESVRPTTINGYYIPAKTRVFINTHGLGRNTSVWTTDIEEFRPERHWPVDGSGRVEISHGPDYKILPFSAGKRKCPGAPLGVTMVLMALARLFHCFDWTTPEDIDTVEVYGMTMPKAKPLWALAKPRLAAHLYTITHDTIGH

SEQ ID NO: 19 - protein, 530 aa, Brassica oleracea
  PEPTID (1)..(530): protein CYPgst (Brassica oleracea)
MDLFLLSIILCSWIFVAVYWKKLNRTKLRLPPGPPRWPIFGNLLQLSPLPHKDFARFCTKYGPLVYLRLGTIDAITTDDPEVIREILIRQDEVFASRPRTLAAVHLAYGCGDVALAPLGPNWKRMRRVCMEHLLTTKRLESFAAHRAQEAEHLCQFVWAKSQSEKPVNLREVLGAFSMNNVTRMLLGKQYFGLQSAGPGEAMEFMHITHELFYLLGLIYLGDYLPAWRWVDPYGCEKKMREVEKKVDDFHQKIIDEHRKAREARKSASSLDDGDDSKEEMDFVDVLLSLPGENGKEHMDDVEIKALMQDMIAAATDTSSVTNEWVMAEVIKHPRVLRKIQEELDAVVGRARMVSESDLPHLPYLRCVVRESFRMHPAGPFLIPHESLKPTTIMGYDIPARTRIFINTHALGRNPRVWDDVGQFRPERHMPADGGARVEISHLPDFKILPFSAGKRKCPGAPLGVILVLMALARLFHCFDWSPPDGEEIDTDEVYGMTMPKALPLFAAARPRLPPEMYHGSSCPSHGKQTM

SEQ ID NO: 20 - protein, 466 aa, Brassica rapa; identical to SEQ ID NO: 18
  PEPTID (1)..(466): protein CYPgst (Brassica rapa)

SEQ ID NO: 21 - protein, 523 aa, Glycine max
  PEPTID (1)..(523): protein CYPgst (Glycine max)
MDLTTFISTLFLGTLASRIIRHWLIGRSLSSHKNKLPPGPPRWPIVGNLLQLGQLPHRDLASLCDKYGPLVYLKLGKIDAITTNDPDIIREILLSQDDVFASRPHTFAAVHLAYGCGDVALAPLGPHWKRMRRICMEHLLTTKRLESFSNHRLDEAQHLVKDVMAWAQDKKPINLREVLGAFSMNNVTRMLLGKQYFGSESSGPQEAMEFMHITHELFWLLGVIYLGDYLPIWRWVDPYGCEKKMREVEKRVDDFHSNIIEEHRKARKDRKGKRKEGDGDMDFVDVLLSLPGEDGKEHMDDVEIKALIQDMIAAATDTSAVTNEWAMAEVMKHPHVLHKIQEELDTIVGPNRMVLESDLPHLNYLRCVVRETFRMHPAGPFLIPHESLRATTINGYHIPAKTRVFINTHGLGRNTKIWDNVDEFRPERHWPSNGNGTRVEISHGVDFKILPFSAGKRKCPGAPLGVTLVLMALARLFHCFDWEPPKGLSCGDVDTREVYGMTMPKAEPLIAIAKPRLAKHLYD

SEQ ID NO: 22 - protein, 537 aa, Gossypium raimondii
  PEPTID (1)..(537): protein CYPgst (Gossypium raimondii)
MIPYKPIFFPLDNMELFTFALALLVGALVVNALWRWRLDWKSLFKTRKLPPGPPRWPIVGNLLQLSSLPHRDLASLCDKYGPLVYLRLGKVDAITTNDPDIIREILLRQDEVFASRPRTLAAVHLAYGCGDVALAPLGPHWKRMRRICMEHLLTTKRLESFAKHRADEAQHLVRDVSARAENGQLVNLREVLGAFSMNNVTRMLLGRQYFGAVSAGPSEAMEFMHITHELFWLLGVIYLGDYLPIWRWVDPYGCEKRMREVEKRVDDFHERIIEEHRRARELKNKGYGKDDDYGEEMDFVDVLLSLPGEDGNPHMDDTDIKALIQDMIAAATDTSAVTNEWTMAEVIKHPRVLRKIQDELDSVVGPNRMVNESDLPHLNYLRCVVRETFRMHPAGPFLIPHESLRATTINGFYIPAKTRVFINTHGLGRNTKLWDDVESFRPERHWLADGARVEISHGADFKILPFSAGKRKCPGAPLGVTLVLMALARLFHCFDWAPQNGMRPEDINTMEVYGMTMPKAEPLMAMAKPRLADHVMF

SEQ ID NO: 23 - protein, 526 aa, Sorghum bicolor
  PEPTID (1)..(526): protein CYPgst (Sorghum bicolor)
MDPFVLSILICSWIFVVVYWRRLNSMRLRLPPGPPTWPIFGNLLQLSPLPHKDFARFCTKYGPLVYLRLGTIDAITTDDPEVIREILIRQDEVFASRPRTLAAVHLAYGCGDVALAPLGPNWKRMRRVCMEHLLTTKRLESFAAHRAQEAEHLCQFVWAKSHSGKPVNLREVLGAFSMNNVTRMLLGKQYFGIQSAGPGEAMEFMHITHELFFLLGLIYLGDYLPAWRWVDPYGCEKKMRDVEKKVDDFHQKIIDEHRRAREAKKTRRSSLDDDDGKEDMDFVDVLLSLPGENGKEHMDDMEIKALMQDMIAAATDTSSVTNEWVMAEVIKNPRVLRRVQEELDAVIGRDRMVAESDLTHLPYLRCVVRESFRMHPAGPFLIPHESLKPTTIMGYHVPARTRVFINTHALGRNPRVWDDVDAFRPERHLPAEEGARVEISHLPDFKILPFSAGKRKCPGAPLGVALVLMALARLFHCFDWSPPDGLRPEDVDTQEVYGMTMPKATPLVAVATPRLPPHLYGGGSAS

SEQ ID NO: 24 - DNA, 41 bp, Artificial Sequence
  sxn2151s01-Markersequenz zum Anzeigen des gst-Locus in Beta vulgaris
aacactcatgtaataagatgggtgagtgagtagcaaaaaaa

SEQ ID NO: 25 - DNA, 41 bp, Artificial Sequence
  sxn2151s01-Markersequenz zum Anzeigen des KWS2320- Referenzgenotyps
aacactcatgtaataagatgagtgagtgagtagcaaaaaaa

SEQ ID NO: 26 - DNA, 41 bp, Artificial Sequence
  sle3305s02-Markersequenz zum Anzeigen des gst-Locus in Beta vulgaris
aaagtctagagtaaattgaggttgcagtggagtgggaagtc

SEQ ID NO: 27 - DNA, 41 bp, Artificial Sequence
  sle3305s02-Markersequenz zum Anzeigen des KWS2320- Referenzgenotyps
aaagtctagagtaaattgagattgcagtggagtgggaagtc